European Patent Application EP 4 560 027 A2, published May 28, 2025. Title: FAST PCR WITH MOLECULAR CROWDING. Applicant: BIOFIRE DEFENSE, LLC. Application EP PCT/US2017/068311, filed December 22, 2017. The sequence listing filed with the application follows.

SEQUENCE LISTING (27 sequences)

SEQ ID NO: 1 - DNA, 24 bp, synthetic construct
  source 1..24: mol_type = other DNA
cccattcaacgtctacatcgagtc

SEQ ID NO: 2 - DNA, 19 bp, synthetic construct
  source 1..19: mol_type = other DNA
tccttctcttgccaggcat

SEQ ID NO: 3 - DNA, 45 bp, Homo sapiens
  variation 26: note = mutation - G or A residue
  source 1..45: mol_type = genomic DNA
cccattcaacgtctacatcgagtccratgcctggcaagagaagga

SEQ ID NO: 4 - DNA, 20 bp, synthetic construct
  source 1..20: mol_type = other DNA
ctacagtgggagtcacctgc

SEQ ID NO: 5 - DNA, 25 bp, synthetic construct
  source 1..25: mol_type = other DNA
ggtactgagctgtgaaagtcaggtt

SEQ ID NO: 6 - DNA, 58 bp, Homo sapiens
  variation 28: note = mutation - A or G residue
  source 1..58: mol_type = genomic DNA
ctacagtgggagtcacctgcttttgccraagggaacctgactttcacagctcagtacc

SEQ ID NO: 7 - DNA, 20 bp, synthetic construct
  source 1..20: mol_type = other DNA
gggagtcacctgcttttgcc

SEQ ID NO: 8 - DNA, 25 bp, synthetic construct
  source 1..25: mol_type = other DNA
tactgagctgtgaaagtcaggttcc

SEQ ID NO: 9 - DNA, 49 bp, Homo sapiens
  source 1..49: mol_type = genomic DNA
gggagtcacctgcttttgccaaagggaacctgactttcacagctcagta

SEQ ID NO: 10 - DNA, 34 bp, synthetic construct
  source 1..34: mol_type = other DNA
ctctgtgctttctgtatcctcagagtggcattct

SEQ ID NO: 11 - DNA, 28 bp, synthetic construct
  source 1..28: mol_type = other DNA
cgtctgctggagtgtgcccaatgctata

SEQ ID NO: 12 - DNA, 60 bp, synthetic construct
  misc_feature 1..41: note = 5' standard synthetic region
  source 1..60: mol_type = other DNA
acacacacacacacacacacacacacacacacacacaaaaattcagtggcattaaatacg

SEQ ID NO: 13 - DNA, 67 bp, synthetic construct
  misc_feature 1..50: note = 5' standard synthetic region
  source 1..67: mol_type = other DNA
gagagagagagagagagagagagagagagagagagagagagagagaaaaaccagagctaaagggaag

SEQ ID NO: 14 - DNA, 66 bp, synthetic construct
  misc_feature 1..41: note = 5' standard synthetic region
  source 1..66: mol_type = other DNA
acacacacacacacacacacacacacacacacacacaaaaagctggtgtctgctatagaactgatt

SEQ ID NO: 15 - DNA, 72 bp, synthetic construct
  misc_feature 1..50: note = 5' standard synthetic region
  source 1..72: mol_type = other DNA
gagagagagagagagagagagagagagagagagagagagagagagaaaaagttgccagagctaaagggaagg

SEQ ID NO: 16 - DNA, 41 bp, synthetic construct
  misc_feature 1..41: note = Synthetic common primer
  source 1..41: mol_type = other DNA
acacacacacacacacacacacacacacacacacacaaaaa

SEQ ID NO: 17 - DNA, 50 bp, synthetic construct
  misc_feature 1..50: note = Synthetic common primer
  source 1..50: mol_type = other DNA
gagagagagagagagagagagagagagagagagagagagagagagaaaaa

SEQ ID NO: 18 - DNA, 24 bp, synthetic construct
  misc_feature 1..24: note = Synthetic common primer
  source 1..24: mol_type = other DNA
actcgcacgaactcaccgcactcc

SEQ ID NO: 19 - DNA, 25 bp, synthetic construct
  misc_feature 1..25: note = Synthetic common primer
  source 1..25: mol_type = other DNA
gctctcactcgcactctcacgcaca

SEQ ID NO: 20 - DNA, 100 bp, synthetic construct
  misc_feature 1..100: note = Synthetic template
  source 1..100: mol_type = other DNA
actcgcacgaactcaccgcactccggatggattgtgaagaggcccaagatactggtcatattatcctttgatctagctctcactcgcactctcacgcaca

SEQ ID NO: 21 - DNA, 200 bp, synthetic construct
  misc_feature 1..200: note = Synthetic template
  source 1..200: mol_type = other DNA
actcgcacgaactcaccgcactcctcaatgctgacaaatcgaaagaataggaatagcgtaattactagaggactccaatatagtatattaccctggtgaccgcctgtactgtaggaacactaccgcggttatattgacagcttagcaatctaccctgttgggatctgtttaagtggctctcactcgcactctcacgcaca

SEQ ID NO: 22 - DNA, 300 bp, synthetic construct
  misc_feature 1..300: note = Synthetic template
  source 1..300: mol_type = other DNA
actcgcacgaactcaccgcactccccttcgaatataaagtacgacattactagcaatgacagttccaggatttaagaaagtagtgttccacatcaatgcatatccagtgaaagcataacgtcaaaaaaagcctggcaccgttcgcgatctggacttacttagatttgttgtagtcaagccggctatcagcgatttatcccggaaacacatactagtgagttatttgtatgttacctagaatagctgtcacgaatcactaatacattcacccaccagctctcactcgcactctcacgcaca

SEQ ID NO: 23 - DNA, 400 bp, synthetic construct
  misc_feature 1..400: note = Synthetic template
  source 1..400: mol_type = other DNA
actcgcacgaactcaccgcactcctgaatacaagacgacagtcctgattatattttcatttaattacgccaatttaattatgatgaatattaacggaattaaatatgtattgataagtactaagtaatggtttacccacggcgatctatatgcaagggaaacattaacaaatttaaacatctgatgtggacaaaacttgtaatgtggtatagttaaaaatataggtttcagggacacgtaagtatctatcttgaatgtttaagtaggtcctgtctaccattctgaaatttagaaaatcgcgttcatcgggctgtcggctacacctcagaaaaccatttcgtgttgcacaggaggaactttcgagggttcgtatgagctctcactcgcactctcacgcaca

SEQ ID NO: 24 - DNA, 500 bp, synthetic construct
  misc_feature 1..500: note = Synthetic template
  source 1..500: mol_type = other DNA
actcgcacgaactcaccgcactccaccgcttgacgacgtagggtatttggtatctgaatctactcatttacctacatactgaagattttgcgatcgtctaatatattggactaatgcccgatttctgatcaattactctaggcgatacttcatcgctggccttatttggattttgctcaagtgctaaactctctgcgcgtcaatactagtctgacatcagtcaagacctgctatctgaaaactactagagagatatacctaacaactttagtggataaatcaggtctggagattgtcatataatgccactagggtcagaaggctgtgtcaaagttagtggttagtaggtctccgctctgcggtactattcttatattctcttactatgcatcaaacaaaatagaatgcatagacaaaccgcctgccaagtttacaagataacttgcgtataggtttataagggttcttctgtatcgctctcactcgcactctcacgcaca

SEQ ID NO: 25 - DNA, 31 bp, synthetic construct
  source 1..31: mol_type = other DNA
gcttggaagattgctaaaatgatagtcagtg

SEQ ID NO: 26 - DNA, 26 bp, synthetic construct
  source 1..26: mol_type = other DNA
ttgatcatactgagcctgctgcataa

SEQ ID NO: 27 - DNA, 60 bp, Homo sapiens
  variation 34: note = mutation - A or G residue
  source 1..60: mol_type = genomic DNA
gcttggaagattgctaaaatgatagtcagtgacrttatgcagcaggctcagtatgatcaa